European Patent Application EP 4 631 545 A1, published October 15, 2025. Title: Method for treating ulceraive colitis or primary sclerosing cholangitis. Applicant: 国立大学法人京都大学. The sequence listing filed with the application follows.

SEQUENCE LISTING (132 sequences)

SEQ ID NO: 1 - protein, 1048 aa, Homo sapiens
MAFPPRRRLRLGPRGLPLLLSGLLLPLCRAFNLDVDSPAEYSGPEGSYFGFAVDFFVPSASSRMFLLVGAPKANTTQPGIVEGGQVLKCDWSSTRRCQPIEFDATGNRDYAKDDPLEFKSHQWFGASVRSKQDKILACAPLYHWRTEMKQEREPVGTCFLQDGTKTVEYAPCRSQDIDADGQGFCQGGFSIDFTKADRVLLGGPGSFYWQGQLISDQVAEIVSKYDPNVYSIKYNNQLATRTAQAIFDDSYLGYSVAVGDFNGDGIDDFVSGVPRAARTLGMVYIYDGKNMSSLYNFTGEQMAAYFGFSVAATDINGDDYADVFIGAPLFMDRGSDGKLQEVGQVSVSLQRASGDFQTTKLNGFEVFARFGSAIAPLGDLDQDGFNDIAIAAPYGGEDKKGIVYIFNGRSTGLNAVPSQILEGQWAARSMPPSFGYSMKGATDIDKNGYPDLIVGAFGVDRAILYRARPVITVNAGLEVYPSILNQDNKTCSLPGTALKVSCFNVRFCLKADGKGVLPRKLNFQVELLLDKLKQKGAIRRALFLYSRSPSHSKNMTISRGGLMQCEELIAYLRDESEFRDKLTPITIFMEYRLDYRTAADTTGLQPILNQFTPANISRQAHILLDCGEDNVCKPKLEVSVDSDQKKIYIGDDNPLTLIVKAQNQGEGAYEAELIVSIPLQADFIGVVRNNEALARLSCAFKTENQTRQVVCDLGNPMKAGTQLLAGLRFSVHQQSEMDTSVKFDLQIQSSNLFDKVSPVVSHKVDLAVLAAVEIRGVSSPDHVFLPIPNWEHKENPETEEDVGPVVQHIYELRNNGPSSFSKAMLHLQWPYKYNNNTLLYILHYDIDGPMNCTSDMEINPLRIKISSLQTTEKNDTVAGQGERDHLITKRDLALSEGDIHTLGCGVAQCLKIVCQVGRLDRGKSAILYVKSLLWTETFMNKENQNHSYSLKSSASFNVIEFPYKNLPIEDITNSTLVTTNVTWGIQPAPMPVPVWVIILAVLAGLLLLAVLVFVMYRMGFFKRVRPPQEEQEREQLQPHENGEGNSET

SEQ ID NO: 2 - protein, 788 aa, Homo sapiens
MGIELLCLFFLFLGRNDHVQGGCALGGAETCEDCLLIGPQCAWCAQENFTHPSGVGERCDTPANLLAKGCQLNFIENPVSQVEILKNKPLSVGRQKNSSDIVQIAPQSLILKLRPGGAQTLQVHVRQTEDYPVDLYYLMDLSASMDDDLNTIKELGSRLSKEMSKLTSNFRLGFGSFVEKPVSPFVKTTPEEIANPCSSIPYFCLPTFGFKHILPLTNDAERFNEIVKNQKISANIDTPEGGFDAIMQAAVCKEKIGWRNDSLHLLVFVSDADSHFGMDSKLAGIVIPNDGLCHLDSKNEYSMSTVLEYPTIGQLIDKLVQNNVLLIFAVTQEQVHLYENYAKLIPGATVGLLQKDSGNILQLIISAYEELRSEVELEVLGDTEGLNLSFTAICNNGTLFQHQKKCSHMKVGDTASFSVTVNIPHCERRSRHIIIKPVGLGDALELLVSPECNCDCQKEVEVNSSKCHHGNGSFQCGVCACHPGHMGPRCECGEDMLSTDSCKEAPDHPSCSGRGDCYCGQCICHLSPYGNIYGPYCQCDNFSCVRHKGLLCGGNGDCDCGECVCRSGWTGEYCNCTTSTDSCVSEDGVLCSGRGDCVCGKCVCTNPGASGPTCERCPTCGDPCNSKRSCIECHLSAAGQAREECVDKCKLAGATISEEEDFSKDGSVSCSLQGENECLITFLITTDNEGKTIIHSINEKDCPKPPNIPMIMLGVSLAILLIGVVLLCIWKLLVSFHDRKEVAKFEAERSKAKWQTGTNPLYRGSTSTFKNVTYKHREKQKVDLSTDC

SEQ ID NO: 3 - protein, 26 aa, Homo sapiens
AKVIPRIRGSGDKAGIKDYYYYGMDV

SEQ ID NO: 4 - protein, 20 aa, Homo sapiens
ATDRPLKLRGRDYNYYVMDV

SEQ ID NO: 5 - protein, 18 aa, Homo sapiens
AKDRGRRGDSGWYRHFDY

SEQ ID NO: 6 - protein, 19 aa, Homo sapiens
ARDRGFRGDTAMIKGGMDV

SEQ ID NO: 7 - protein, 4 aa, Homo sapiens
RGRD

SEQ ID NO: 8 - protein, 5 aa, Homo sapiens
RGSGD

SEQ ID NO: 9 - protein, 4 aa, synthetic construct
RGDS

SEQ ID NO: 10 - protein, 4 aa, synthetic construct
RGES

SEQ ID NO: 11 - protein, 8 aa, Homo sapiens
GFTFSSYG

SEQ ID NO: 12 - protein, 8 aa, Homo sapiens
ISYDGINK

SEQ ID NO: 13 - protein, 26 aa, Homo sapiens
AKVIPRIRGSGDKAGIKDYYYYGMDV

SEQ ID NO: 14 - protein, 11 aa, Homo sapiens
QNLLHSNGYNY

SEQ ID NO: 15 - skipped

SEQ ID NO: 16 - protein, 8 aa, Homo sapiens
MQALQTWT

SEQ ID NO: 17 - protein, 8 aa, Homo sapiens
GFTITNAW

SEQ ID NO: 18 - protein, 10 aa, Homo sapiens
SKSKTDGGTT

SEQ ID NO: 19 - protein, 20 aa, Homo sapiens
ATDRPLKLRGRDYNYYVMDV

SEQ ID NO: 20 - protein, 6 aa, Homo sapiens
QSIARS

SEQ ID NO: 21 - skipped

SEQ ID NO: 22 - protein, 9 aa, Homo sapiens
QQSSSSPLT

SEQ ID NO: 23 - protein, 8 aa, Homo sapiens
GFTFSIYG

SEQ ID NO: 24 - protein, 8 aa, Homo sapiens
ISSDGTNQ

SEQ ID NO: 25 - protein, 18 aa, Homo sapiens
AKDRGRRGDSGWYRHFDY

SEQ ID NO: 26 - protein, 8 aa, Homo sapiens
SSNNGNNY

SEQ ID NO: 27 - skipped

SEQ ID NO: 28 - protein, 11 aa, Homo sapiens
GTWDSSLSAVV

SEQ ID NO: 29 - protein, 8 aa, Homo sapiens
GYTFSSFG

SEQ ID NO: 30 - protein, 8 aa, Homo sapiens
ISAYNGNT

SEQ ID NO: 31 - protein, 19 aa, Homo sapiens
ARDRGFRGDTAMIKGGMDV

SEQ ID NO: 32 - protein, 6 aa, Homo sapiens
ALPKQY

SEQ ID NO: 33 - skipped

SEQ ID NO: 34 - protein, 10 aa, Homo sapiens
SSTDSNSQRV

SEQ ID NO: 35 - protein, 8 aa, Homo sapiens
GHTFSSFG

SEQ ID NO: 36 - protein, 8 aa, Homo sapiens
ISAYNGNT

SEQ ID NO: 37 - protein, 19 aa, Homo sapiens
ARDRGFRGDTAMIKGGMDV

SEQ ID NO: 38 - protein, 6 aa, Homo sapiens
KLGDKY

SEQ ID NO: 39 - skipped

SEQ ID NO: 40 - protein, 10 aa, Homo sapiens
QAWDSSTALV

SEQ ID NO: 41 - protein, 8 aa, Homo sapiens
GHTFSSFG

SEQ ID NO: 42 - protein, 8 aa, Homo sapiens
ISAYNGNT

SEQ ID NO: 43 - protein, 19 aa, Homo sapiens
ARDRGFRGDTAMIKGGMDV

SEQ ID NO: 44 - protein, 9 aa, Homo sapiens
SSTIGANND

SEQ ID NO: 45 - skipped

SEQ ID NO: 46 - protein, 12 aa, Homo sapiens
QSYDSSLSDLYV

SEQ ID NO: 47 - protein, 8 aa, Homo sapiens
GFTFSSYG

SEQ ID NO: 48 - protein, 8 aa, Homo sapiens
ISYDGINK

SEQ ID NO: 49 - protein, 26 aa, Homo sapiens
AKVIPRIRGSGDKAGIKDYYYYGMDV

SEQ ID NO: 50 - protein, 6 aa, Homo sapiens
QSVSSY

SEQ ID NO: 51 - skipped

SEQ ID NO: 52 - protein, 8 aa, Homo sapiens
QQRSNWLT

SEQ ID NO: 53 - protein, 8 aa, Homo sapiens
GFTFSSYA

SEQ ID NO: 54 - protein, 8 aa, Homo sapiens
ISYDGINK

SEQ ID NO: 55 - protein, 26 aa, Homo sapiens
AKVIPRIRGSGDKAGIKDYYYYGMDV

SEQ ID NO: 56 - protein, 7 aa, Homo sapiens
QSVSSSY

SEQ ID NO: 57 - skipped

SEQ ID NO: 58 - protein, 9 aa, Homo sapiens
QQYGSSVWT

SEQ ID NO: 59 - protein, 8 aa, Homo sapiens
GFTFSSYG

SEQ ID NO: 60 - protein, 8 aa, Homo sapiens
ISYDGINK

SEQ ID NO: 61 - protein, 26 aa, Homo sapiens
AKVIPRIRGSGDKAGIKDYYYYGMDV

SEQ ID NO: 62 - protein, 8 aa, Homo sapiens
SSNIGNNY

SEQ ID NO: 63 - skipped

SEQ ID NO: 64 - protein, 11 aa, Homo sapiens
GTWDSSLSAVV

SEQ ID NO: 65 - protein, 9 aa, Homo sapiens
GYTLTELRI

SEQ ID NO: 66 - protein, 9 aa, Homo sapiens
DPEDGETIY

SEQ ID NO: 67 - protein, 17 aa, Homo sapiens
TTDLFAFVRGVRGAFDI

SEQ ID NO: 68 - protein, 6 aa, Homo sapiens
TITTYL

SEQ ID NO: 69 - protein, 5 aa, Homo sapiens
ASSLH

SEQ ID NO: 70 - protein, 9 aa, Homo sapiens
QQSYRTLWT

SEQ ID NO: 71 - protein, 8 aa, Homo sapiens
GHTFSSFG

SEQ ID NO: 72 - protein, 8 aa, Homo sapiens
ISAYNGNT

SEQ ID NO: 73 - protein, 19 aa, Homo sapiens
ARDRGFRGDTAMIKGGMDV

SEQ ID NO: 74 - protein, 9 aa, Homo sapiens
SSDVGGYNY

SEQ ID NO: 75 - skipped

SEQ ID NO: 76 - protein, 10 aa, Homo sapiens
SSYTSSSTYV

SEQ ID NO: 77 - protein, 8 aa, Homo sapiens
GFDFSNYV

SEQ ID NO: 78 - protein, 8 aa, Homo sapiens
ITDRGDSR

SEQ ID NO: 79 - protein, 16 aa, Homo sapiens
AKDQTFAGDDPTVFDS

SEQ ID NO: 80 - protein, 9 aa, Homo sapiens
SSDIGGYNY

SEQ ID NO: 81 - skipped

SEQ ID NO: 82 - protein, 10 aa, Homo sapiens
NSYTTSSTSV

SEQ ID NO: 83 - protein, 133 aa, Homo sapiens
QVQLVESGGGVVQPGRSLRLSCAASGFTFSSYGMHWVRQAPGKGLEWVAFISYDGINKYYADSVKGRFTISRDNSKDTLYLQMNSLRAEDTAVYYCAKVIPRIRGSGDKAGIKDYYYYGMDVWGQGTTVTVSS

SEQ ID NO: 84 - protein, 111 aa, Homo sapiens
DIVMTQSPLSLPVTPGEPASISCRSSQNLLHSNGYNYLDWYLQKPGQSPQLLIYLGSNRASGVPDRFSGSGSGTDFTLKISRVEAEDVGVYYCMQALQTWTFGQGTKVEIK

SEQ ID NO: 85 - protein, 129 aa, Homo sapiens
EVQLVESGGGLVKPGGSLRVSCVVSGFTITNAWMSWVRQAPGKGLEWVGRSKSKTDGGTTDYIAPVKGRFTISRDDSKNTLYLEMNSLKTEDTAVYYCATDRPLKLRGRDYNYYVMDVWGQGTTVTVSS

SEQ ID NO: 86 - protein, 107 aa, Homo sapiens
DIQMTQSPSSLSASVGDRVTITCRASQSIARSLNWYQQKPGKAPNLLIYAASTLQSGVPSRFSGSGSGTDFTLTIGSLQPEDFATYSCQQSSSSPLTFGGGTRVEIK

SEQ ID NO: 87 - protein, 125 aa, Homo sapiens
QVQLVESGGGVVQPGRSLRVSCAASGFTFSIYGMHWVRQAPGKGLEWVAVISSDGTNQYYADSVKGRFTISRDNSNNTVYLQMNSLGGEDTAVYYCAKDRGRRGDSGWYRHFDYWGQGTLVTVSS

SEQ ID NO: 88 - protein, 110 aa, Homo sapiens
QSVLTQPPSVSAAPGQKVTISCSGSSSNNGNNYVSWYQQVPGTAPKLLIYDNNKRPSGIPDRFSGSKSGTSATLGITGLQTGDEADYYCGTWDSSLSAVVFGGGTKLTVL

SEQ ID NO: 89 - protein, 126 aa, Homo sapiens
QVQLVQSGAEVKKPGASVKVSCKASGYTFSSFGISWVRQAPGQGLEWMGWISAYNGNTNSAQKFQGRVTMTTDTSTSTAYMELRSLRSDDTAVYYCARDRGFRGDTAMIKGGMDVWGQGTTVTVSS

SEQ ID NO: 90 - protein, 107 aa, Homo sapiens
SYELTQPPSVSVSPGQTARITCSGDALPKQYAYWYQQKPGQAPVLVIYKDSERPSGIPERFSGSSSGTMATLTISGAQVEDEGDYYCSSTDSNSQRVFGGGTKLTVL

SEQ ID NO: 91 - protein, 126 aa, Homo sapiens
QVQLVQSGAEVKKPGASVKVSCKASGHTFSSFGISWVRQAPGQGLEWMGWISAYNGNTNSAQKFQGRVTMTTDTSTSTAYMELRSLRSDDTAVYYCARDRGFRGDTAMIKGGMDVWGQGTTVTVSS

SEQ ID NO: 92 - protein, 105 aa, Homo sapiens
VLTQPPSVSVSPGQTASITCSGDKLGDKYACWYQQKSGQAPVLVIYQDSKRPSGIPERFSGSNSGNTATLTISGTQAMDEADYYCQAWDSSTALVFGGGTKLTVL

SEQ ID NO: 93 - protein, 126 aa, Homo sapiens; identical to SEQ ID NO: 91

SEQ ID NO: 94 - protein, 112 aa, Homo sapiens
QSVLTQPPSVSGAPGQRVTISCTGSSSTIGANNDVHWYQQLPGTAPKLLIYGNKNRPSGVSDRFSGSKSGTSASLAITGLQAEDEADYYCQSYDSSLSDLYVFGTGTKVTVL

SEQ ID NO: 95 - protein, 132 aa, Homo sapiens
VQLVESGGGVVQPGRSLRLSCAASGFTFSSYGMHWVRQAPGKGLEWVAFISYDGINKYYADSVKGRFTISRDNSKDTLYLQMNSLRAEDTAVYYCAKVIPRIRGSGDKAGIKDYYYYGMDVWGQGTTVTVSS

SEQ ID NO: 96 - protein, 106 aa, Homo sapiens
EIVLTQSPATLSLSPGERATLSCRASQSVSSYLAWYQQKPGQAPRLLIYDASNRATGIPARFSGSGSGTDFTLTISSLEPEDFAVYYCQQRSNWLTFGGGTKVEIK

SEQ ID NO: 97 - protein, 133 aa, Homo sapiens
QVQLVESGGGVVQPGRSLRLSCAASGFTFSSYAMHWVRQAPGKGLEWVAFISYDGINKYYADSVKGRFTISRDNPKDTLYLQMNSLRAEDTAVYYCAKVIPRIRGSGDKAGIKDYYYYGMDVWGRGTTVTVSS

SEQ ID NO: 98 - protein, 108 aa, Homo sapiens
EIVLTQSPGTLSLSPGERATLSCRASQSVSSSYLAWYQQKPGQAPRLLIYGASSRATGIPDRFSGSGSGTDFTLTISRLEPEDFAVYYCQQYGSSVWTFGQGTKVEIK

SEQ ID NO: 99 - protein, 133 aa, Homo sapiens; identical to SEQ ID NO: 83

SEQ ID NO: 100 - protein, 110 aa, Homo sapiens
QSVLTQPPSVSAAPGQKVTISCSGSSSNIGNNYVSWYQQLPGTAPKLLIYDNNKRPSGIPDRFSGSKSGTSATLGITGLQTGDEADYYCGTWDSSLSAVVFGGGTKLTVL

SEQ ID NO: 101 - protein, 124 aa, Homo sapiens
QVQLVQSGAEVKKPGASVKVSCKVSGYTLTELRIHWVRQVPGKGLEWMGGFDPEDGETIYTQKFQGRVTMTEDTSTDTAYMELSSLRSEDTAVYYCTTDLFAFVRGVRGAFDIWGQGTMVTVSS

SEQ ID NO: 102 - protein, 107 aa, Homo sapiens
DIQMTQSPSSLSASVGDRVTITCRASQTITTYLNWYQQKPGKAPKLLIYRASSLHSGVPSRFSGSGSGTDFTLTISSLQPEDFATYYCQQSYRTLWTFGQGTKVEIN

SEQ ID NO: 103 - protein, 126 aa, Homo sapiens; identical to SEQ ID NO: 91

SEQ ID NO: 104 - protein, 110 aa, Homo sapiens
QSALTQPASVSGSPGQSITISCTGTSSDVGGYNYVSWYQQHPGKAPQLIIYDVSKRPSGVSNRFSGSRSGNTASLTISGLQAEDEADYYCSSYTSSSTYVFGTGTKVTVL

SEQ ID NO: 105 - protein, 123 aa, Homo sapiens
EAHLLESGGGLVQPGGSLRLSCEGSGFDFSNYVMNWVRQAPGKGLEWVSAITDRGDSRYYINSVKGRFTISRDNSKNTLFLEMYGLTPEDTAVYYCAKDQTFAGDDPTVFDSWGLGTLVTVSS

SEQ ID NO: 106 - protein, 110 aa, Homo sapiens
QSALTQPASVSGSPGQSITISCTGTSSDIGGYNYVSWYQQHPGKAPKLMIYDVNKRPSGVSNRFSGSKSGNTASLTISGLQAEDEADYYCNSYTTSSTSVFGTGTKVTVL

SEQ ID NO: 107 - DNA, 399 bp, Homo sapiens
  source 1..399: mol_type = genomic DNA
caggtgcagctggtggagtctgggggaggcgtggtccagcctgggaggtccctgagactctcctgtgcagcctctggattcaccttcagtagctatggcatgcactgggtccgccaggctccaggcaaggggctggagtgggtggcatttatatcatatgatggaattaataaatactatgcagactccgtgaagggccgcttcaccatctccagagacaattccaaggacacgctgtatctgcaaatgaacagcctgagagctgaggacacggctgtatattactgtgcgaaagtcatccccaggataaggggttcgggagacaaagcggggataaaagactactactactacggtatggacgtctggggccaagggaccacggtcaccgtctcctca

SEQ ID NO: 108 - DNA, 333 bp, Homo sapiens
  source 1..333: mol_type = genomic DNA
gatattgtgatgactcagtctccactctccctgcccgtcacccctggagagccggcctccatctcctgcaggtctagtcagaacctcctgcatagtaatggatacaactatttggattggtacctgcagaagccagggcagtctccacagctcctgatctatttgggttctaatcgggcctccggggtccctgacaggttcagtggcagtggatcaggcacagattttacactgaaaatcagcagagtggaggctgaggatgttggggtttattactgcatgcaagctctacaaacttggacgttcggccaagggaccaaggtggaaatcaaa

SEQ ID NO: 109 - DNA, 387 bp, Homo sapiens
  source 1..387: mol_type = genomic DNA
gaggtgcagttggtggagtctgggggaggcttggtaaagcctggggggtcccttagagtctcctgtgtagtctctggattcacaatcactaacgcctggatgagctgggtccgccaggctccagggaaggggctggagtgggttggccgtagtaaaagcaaaactgatggtgggacaacagactacattgcacccgtgaaaggcagattcaccatctcaagagatgattcaaaaaacacactttatctggaaatgaacagcctgaaaaccgaggacacagccgtgtattactgtgccacagatcggcctctgaaactaaggggtagagactacaactactacgttatggacgtctggggccaagggaccacggtcaccgtctcctca

SEQ ID NO: 110 - DNA, 321 bp, Homo sapiens
  source 1..321: mol_type = genomic DNA
gacatccagatgacccagtctccatcctccctgtctgcttctgttggagacagagtcaccatcacttgccgggcaagtcagagcattgccagatctttaaattggtatcagcaaaaaccagggaaagcccctaatctcctgatctatgctgcatccactttgcaaagtggggtcccatcaaggttcagtggcagtggatctgggacagatttcactctcaccatcggcagtctgcaacctgaagatttcgcaacttactcctgtcaacagagttccagttcccctctcactttcggcggagggaccagggtggagatcaag

SEQ ID NO: 111 - DNA, 375 bp, Homo sapiens
  source 1..375: mol_type = genomic DNA
caggtgcagctggtggagtctgggggaggcgtggtccagcctgggaggtccctgagagtctcctgtgcagcctctggattcaccttcagtatttatgggatgcactgggtccgccaggctccaggcaaggggctggagtgggtggcagttatttcatctgatggaactaatcaatactatgcagactccgtgaagggccgattcaccatctccagagacaattccaacaacacggtgtatctgcaaatgaacagcctgggaggtgaggacacggctgtgtattactgtgcgaaagatcggggccgccggggggacagtggctggtaccgacactttgactactggggccagggaaccctggtcaccgtctcctca

SEQ ID NO: 112 - DNA, 330 bp, Homo sapiens
  source 1..330: mol_type = genomic DNA
cagtctgtgttgacgcagccgccctcagtgtctgcggccccaggacagaaggtcaccatctcctgctctggaagcagctccaacaatgggaataattatgtatcctggtaccagcaggtcccaggaacagcccccaaactcctcatttatgacaataataagcgaccctcagggattcctgaccgattctctggctccaagtctggcacgtcagccaccctgggcatcaccggactccagactggggacgaggccgattattactgcggaacatgggatagcagcctgagtgctgtagtcttcggcggagggaccaagctgaccgtccta

SEQ ID NO: 113 - DNA, 378 bp, Homo sapiens
  source 1..378: mol_type = genomic DNA
caggttcagctggtgcagtctggagctgaggtgaagaagcctggggcctcagtgaaggtctcctgcaaggcttctggttacaccttttccagctttggtatcagctgggtgcgacaggcccctggacaagggcttgagtggatgggatggatcagcgcttacaatggtaacacaaactctgcacagaagttccagggcagagtcaccatgaccacagacacatccacgagcacagcctacatggagctgaggagcctgagatctgacgacacggccgtgtattactgtgcgagagataggggttttcgcggggacacagctatgattaaagggggtatggacgtctggggccaagggaccacggtcaccgtctcctca

SEQ ID NO: 114 - DNA, 321 bp, Homo sapiens
  source 1..321: mol_type = genomic DNA
tcctatgagctgacacagccaccctcggtgtcagtgtccccaggacagacggccaggatcacctgctctggagatgcattgccaaagcaatatgcttattggtaccagcagaagccaggccaggcccctgtgctggtgatatataaagacagtgagaggccctcagggatccctgagcgattctctggctccagctcagggacaatggccaccttgactatcagtggggcccaggtggaggatgaaggtgactactactgttcctcaacagacagcaattctcagcgcgtattcggcggagggaccaagctgaccgtccta

SEQ ID NO: 115 - DNA, 378 bp, Homo sapiens
  source 1..378: mol_type = genomic DNA
caggttcagctggtgcagtctggagctgaggtgaagaagcctggggcctcagtgaaggtctcctgcaaggcttctggtcacaccttttccagctttggtatcagctgggtgcgacaggcccctggacaagggcttgagtggatgggatggatcagcgcttacaatggtaacacaaactctgcacagaagttccagggcagagtcaccatgaccacagacacatccacgagcacagcctacatggagctgaggagcctgagatctgacgacacggccgtgtattactgtgcgagagataggggttttcgcggggacacagctatgattaaagggggtatggacgtctggggccaagggaccacggtcaccgtctcctca

SEQ ID NO: 116 - DNA, 315 bp, Homo sapiens
  source 1..315: mol_type = genomic DNA
gtgctgacgcagccgccctcagtgtccgtgtccccaggacagacagccagcatcacctgctctggagataaattgggggataaatatgcttgctggtaccagcagaagtcaggccaggcccctgtattggtcatctatcaagatagcaagcggccctcagggatccctgagcgattctctggctccaactctgggaacacagccactctgaccatcagcgggacccaggctatggatgaggctgactattactgtcaggcgtgggacagcagcactgcgctggtattcggcggagggaccaagctgaccgtccta

SEQ ID NO: 117 - DNA, 378 bp, Homo sapiens; identical to SEQ ID NO: 115
  source 1..378: mol_type = genomic DNA

SEQ ID NO: 118 - DNA, 336 bp, Homo sapiens
  source 1..336: mol_type = genomic DNA
cagtctgtgctgacgcagccgccctcagtgtctggggccccagggcagagggtcaccatctcctgcactgggagcagttccaccatcggggcaaataatgatgtacactggtaccagcaacttccaggaacagcccccaaactcctcatctatggtaacaagaatcgcccctcaggggtctctgaccgattctctggctccaagtctggcacctcagcctccctggccatcactgggctccaggctgaggatgaggctgattattactgccagtcctatgacagcagtctgagtgatctttatgtcttcggaacggggaccaaggtcaccgtccta

SEQ ID NO: 119 - DNA, 396 bp, Homo sapiens
  source 1..396: mol_type = genomic DNA
gtgcagctggtggagtctggaggaggcgtggtccagcctgggaggtccctgagactctcctgtgcagcctctggattcaccttcagtagctatggcatgcactgggtccgccaggctccaggcaaggggctggagtgggtggcatttatatcatatgatggaattaataaatactatgcagactccgtgaagggccgcttcaccatctccagagacaattccaaggacacgctgtatctgcaaatgaacagcctgagagctgaggacacggctgtatattactgtgcgaaagtcatccccaggataaggggttcgggagacaaagcggggataaaagactactactactacggtatggacgtctggggccaagggaccacggtcaccgtctcctca

SEQ ID NO: 120 - DNA, 318 bp, Homo sapiens
  source 1..318: mol_type = genomic DNA
gaaattgtgttgacacagtctccagccaccctgtctttgtctccaggggaaagagccaccctctcctgcagggccagtcagagtgttagcagctacttagcctggtaccaacagaaacctggccaggctcccaggctcctcatctatgatgcatccaacagggccactggcatcccagccaggttcagtggcagtgggtctgggacagacttcactctcaccatcagcagcctagagcctgaagattttgcagtttattactgtcagcagcgtagcaactggctcactttcggcggagggaccaaggtggagatcaaa

SEQ ID NO: 121 - DNA, 399 bp, Homo sapiens
  source 1..399: mol_type = genomic DNA
caggtgcagctggtggagtctgggggaggcgtggtccaacctgggaggtccctgagactctcctgtgcagcctctggattcaccttcagtagctatgctatgcactgggtccgccaggctccaggcaaggggctggagtgggtggcatttatatcatatgatggaattaataaatactatgcagactccgtgaagggccgcttcaccatctccagagacaatcccaaggacacgctgtatctgcaaatgaacagcctgagagctgaggacacggctgtatattactgtgcgaaagtcatccccaggataaggggttcgggagacaaagcggggataaaagactactactactacggtatggacgtctggggccgagggaccacggtcaccgtctcctca

SEQ ID NO: 122 - DNA, 324 bp, Homo sapiens
  source 1..324: mol_type = genomic DNA
gaaattgtgttgacacagtctccaggcaccctgtctttgtctccaggggaaagagccaccctctcctgcagggccagtcagagtgttagcagcagctacttagcctggtaccagcagaaacctggccaggctcccaggctcctcatctatggtgcatccagcagggccactggcatcccagacaggttcagtggcagtgggtctgggacagacttcactctcaccatcagcagactggagcctgaagattttgcagtgtattactgtcagcagtatggtagctcagtgtggacgttcggccaagggaccaaggtggaaatcaaa

SEQ ID NO: 123 - DNA, 399 bp, Homo sapiens; identical to SEQ ID NO: 107
  source 1..399: mol_type = genomic DNA

SEQ ID NO: 124 - DNA, 330 bp, Homo sapiens
  source 1..330: mol_type = genomic DNA
cagtctgtgttgacgcagccgccctcagtgtctgcggccccaggacagaaggtcaccatctcctgctctggaagcagctccaacattgggaataattatgtatcctggtaccagcagctcccaggaacagcccccaaactcctcatttatgacaataataagcgaccctcagggattcctgaccgattctctggctccaagtctggcacgtcagccaccctgggcatcaccggactccagactggggacgaggccgattattactgcggaacatgggatagcagcctgagtgctgtggtattcggcggagggaccaagctgaccgtccta

SEQ ID NO: 125 - DNA, 372 bp, Homo sapiens
  source 1..372: mol_type = genomic DNA
caggtccagctggtacagtctggggctgaggtgaagaagcctggggcctcagtgaaagtctcctgcaaggtttccggatacaccctcactgaattacgcatacactgggtgcgacaggttcctggaaaagggcttgagtggatgggaggttttgatcctgaagatggtgaaacaatctacacacagaagttccagggcagagtcacgatgaccgaggacacatctacagacacagcctacatggagctgagcagcctgagatctgaggacacggccgtctattactgtacaacagatcttttcgctttcgttcggggagttaggggtgcttttgatatctggggccaggggacaatggtcaccgtctcttca

SEQ ID NO: 126 - DNA, 321 bp, Homo sapiens
  source 1..321: mol_type = genomic DNA
gacatccagatgacccagtctccatcctccctgtctgcatctgtaggagacagagtcaccatcacttgccgggcaagtcagaccattactacttatttaaattggtatcagcagaaaccagggaaagcccctaagctcctgatctatagagcatccagtttgcacagtggggtcccatctaggttcagtggcagtggatctgggacagatttcactctcaccatcagcagtctgcaacctgaagattttgcaacttactactgtcaacagagttaccgtaccctctggacgttcggccaagggaccaaggtggaaatcaac

SEQ ID NO: 127 - DNA, 378 bp, Homo sapiens; identical to SEQ ID NO: 115
  source 1..378: mol_type = genomic DNA

SEQ ID NO: 128 - DNA, 330 bp, Homo sapiens
  source 1..330: mol_type = genomic DNA
cagtctgccctgactcagcctgcctccgtgtctgggtctcctggacagtcgatcaccatctcctgcactggaaccagcagtgacgttggtggttataactatgtctcctggtaccaacagcacccaggcaaagccccccaactcataatttatgatgtcagtaagcggccctcaggggtttctaatcgcttctctggctccaggtctggcaacacggcctccctgaccatctctgggctccaggctgaggacgaggctgattattactgcagctcatatacaagcagcagcacttatgtcttcggaactgggaccaaggtcaccgtccta

SEQ ID NO: 129 - DNA, 369 bp, Homo sapiens
  source 1..369: mol_type = genomic DNA
gaggcgcatctgttggagtctgggggaggcctggtacagcctggggggtccctgagactctcatgtgaaggctctgggttcgactttagcaattatgtcatgaactgggtccgccaggctccagggaaggggctggagtgggtctccgcaattactgacagaggtgatagtcgatactatataaattcagtgaagggccggttcaccatctccagagacaattccaagaacacgctgtttctggagatgtacggcctgacacccgaagacacggccgtctattactgtgccaaggatcagacatttgcgggcgacgaccccaccgtcttcgactcctggggcctgggaaccctggtcaccgtctcctca

SEQ ID NO: 130 - DNA, 330 bp, Homo sapiens
  source 1..330: mol_type = genomic DNA
cagtctgccctgactcagcctgcctccgtgtctgggtctcctggacagtcgatcaccatctcctgcactggaaccagcagtgacattggtggttataactatgtctcctggtaccaacaacacccaggcaaagcccccaaactcatgatttatgatgtcaataagcggccctcaggggtttctaatcgcttctctggctccaagtctggcaacacggcctccctgaccatctctgggctccaggctgaggacgaggctgattattactgcaactcatatacaaccagcagcacttctgtcttcggaactgggaccaaggtcaccgtccta

SEQ ID NO: 131 - protein, 10 aa, synthetic construct
GGGGSGGGGS

SEQ ID NO: 132 - protein, 5 aa, synthetic construct
GGGGS